European Patent Specification EP 3 874 269 B1, published March 11, 2026. Title: Sensor. Applicant: University of the West of England. The sequence listing filed with the application follows.

SEQUENCE LISTING (37 sequences)

SEQ ID NO: 1 - DNA, 1002 bp, Artificial Sequence
  Recombinant CSSV coat protein antigen 01
gttgactatacaccacctggtgacacactgatgacacctgtcggatatccaccggcctcgtcatcaagatcaacagtaacaacaccaagtaggccccctttatttgaaggaagggttacacacgtgccaagattcttaaaacgggatgactacacagaatggtggcaactaccatcatcccaaggcacaactggggcattatttgtgatgcccaaacaaataggcctatttcatgatgtcttctccagatgggagtccatcaccaaaaactatgttgcggcccaaagtttcacggacccaacagaaaagatggagttcatggaaaacttacttggagaaacagaaaaactaacctggatccaatggagaatgaattatgaggctgagtaccagcagctgttaacccaagctgatggacggcaagggacccagaatatcttgtcccaaattaagagagtcttctctctagaagaccccgcctcaggatccacgaggatacaagatgctgcatacagagaccttgaaagattgacctgccacaacataaaagatatcgttcagttcctgaatgattatgggcggttagcagcaaaaagtgggcgactgtttctaggaacagagctcagtgaaaaactatggatgaagatgccaccagaactagggaatcgcatgaaggaagcatttcaaaaggaatactcaggcaatgaagtaggagtcttcccgcgtatcttgttcgcgtacagatacttagaacaagaatgcaaagatgcagcgtttaagcgcagcctgaagtcgttgagtttctgtaaggacatgccgttgacaggttactatgataaaacacccaaatacggcatgaggaagtcaaaaacttacaaaggaaagccacacgcatcacatgcaagagtagaaaagagaaagcacttaatcaggaataaaaagtgcaagtgctatctgtgtggagatgaaggacattttgccagagaatgccctaataacaaa

SEQ ID NO: 2 - protein, 334 aa, Artificial Sequence
  Recombinant CSSV coat protein antigen 01 putative amino acid sequence
VDYTPPGDTLMTPVGYPPASSSRSTVTTPSRPPLFEGRVTHVPRFLKRDDYTEWWQLPSSQGTTGALFVMPKQIGLFHDVFSRWESITKNYVAAQSFTDPTEKMEFMENLLGETEKLTWIQWRMNYEAEYQQLLTQADGRQGTQNILSQIKRVFSLEDPASGSTRIQDAAYRDLERLTCHNIKDIVQFLNDYGRLAAKSGRLFLGTELSEKLWMKMPPELGNRMKEAFQKEYSGNEVGVFPRILFAYRYLEQECKDAAFKRSLKSLSFCKDMPLTGYYDKTPKYGMRKSKTYKGKPHASHARVEKRKHLIRNKKCKCYLCGDEGHFARECPNNK

SEQ ID NO: 3 - DNA, 990 bp, Artificial Sequence
  recombinant CSSV coat protein antigen 02 DNA sequence
gttgactacacacctcctggagatacgttaatgactccagttgggtatccacctgcatcaacatctagacaaccacaaccgtctagacccccactgtatgagggacgaatccctcagattcctagattcagaaaagatgactacactgaatggtggcaattgccatcttcgcaagccacaacaggagccttatttgttatgccaaagcaaattggcttcttccatgacgtcttttccagatgggaatcagtcacgaagaactacatagctttgcaggagttcactgatcctgctgacaaagttgaattcatagaaaacctgctgggagaaacagaaaagctaacatggattcaatggaggatgaactatgtagcagaatatcagcaactgataacacaagctgatggaagacaagggacacagaatatcctgtcccaaataaagagaatcttctctttagaagaccctgcatcagggtctacaaggatacaagatgctgcttacagagatctggagagattaacatgcaacaacatcaaagacatagtccaattcctgaatgactatggcagattagcagcaaaaactggcagaatgttcataagcagagagcttagtgataaactatggctcaaaatgccgccagaactgggaaccagaatgaaggaagcgtatgacaaggagtacccaggcaatgacgtaggagtatatcccagaatactctacgcctacaaatacctggaacaggagtgtaaagacgcagccttcaaaagaagtctgaaatctctgagtttctgcagagatataccaatcaccgggtactacgacaagccaaagtatggtgtccggagatccactacatacaaaggaaagccacatgcaacacatgcaaggattgaaaagaagaaacacctagtcagaaacaaaaggtgtaaatgttatttatgtggcgatgaaggccattttgctagagaatgccctaatgcaaaa

SEQ ID NO: 4 - protein, 330 aa, Artificial Sequence
  recombinant CSSV coat protein antigen 02 - putative amino acid sequence
VDYTPPGDTLMTPVGYPPASTSRQPQPSRPPLYEGRIPQIPRFRKDDYTEWWQLPSSQATTGALFVMPKQIGFFHDVFSRWESVTKNYIALQEFTDPADKVEFIENLLGETEKLTWIQWRMNYVAEYQQLITQADGRQGTQNILSQIKRIFSLEDPASGSTRIQDAAYRDLERLTCNNIKDIVQFLNDYGRLAAKTGRMFISRELSDKLWLKMPPELGTRMKEAYDKEYPGNDVGVYPRILYAYKYLEQECKDAAFKRSLKSLSFCRDIPITGYYDKPKYGVRRSTTYKGKPHATHARIEKKKHLVRNKRCKCYLCGDEGHFARECPNAK

SEQ ID NO: 5 - protein, 690 aa, Artificial Sequence
  AbD31988 - Amino acid sequence of Fd chain and tags
QVQLVQSGAEVKKPGASVKVSCKASGYTFSNYYMSWVRQAPGQGLEWMGWINPYNGVTNYAQKFQGRVTMTRDTSISTAYMELSRLRSEDTAVYYCARGLGSQFDYWGQGTLVTVSSASTKGPSVFPLAPSSKSTSGGTAALGCLVKDYFPEPVTVSWNSGALTSGVHTFPAVLQSSGLYSLSSVVTVPSSSLGTQTYICNVNHKPSNTKVDKKVEPKSEFKAEMPVLENRAAQGDITTPGGARRLTGDQTAALRDSLSDKPAKNIILLIGDGMGDSEITAARNYAEGAGGFFKGIDALPLTGQYTHYALNRKTGKPDYVTSSAASATAWSTGVKTYNGALGVDIHEKDHPTILEMAKAAGLATGNVSTAELQDATPAALVAHVTSRKCYGPSATSEKCPGNALEKGGKGSITEQLLNARADVTLGGGAKTFAETATAGEWQGKTLREQAQARGYQLVSDAASLNSVTEANQQKPLLGLFADGNMPVRWLGPKATYHGNIDKPAVTCTPNFQRNDSVPTLAQMTDKAIELLSKNEKGFFLQVEGASIDKQDHAANPCGQIGETVDLDEAVQRALEFAKKEGNTLVIVTADHAHASQIVAPDTKAPGLTQALNTKDGAVMVMSYGNSEEDSQEHTGSQLRIAAYGPHAANVVGLTDQTDLFYTMKAALGLKGAPDYKDDDDKGAPHHHHHH

SEQ ID NO: 6 - protein, 221 aa, Artificial Sequence
  AbD31988 heavy chain
QVQLVQSGAEVKKPGSSVKVSCKASGGTFSSYAISWVRQAPGQGLEWMGRIIPIFGTANYAQKFQGRVTITADESTSTAYMELSSLRSEDTAVYYCARGGYRYFDIWGQGTLVTVSSASTKGPSVFPLAPSSKSTSGGTAALGCLVKDYFPEPVTVSWNSGALTSGVHTFPAVLQSSGLYSLSSVVTVPSSSLGTQTYICNVNHKPSNTKVDKKVEPKSEF

SEQ ID NO: 7 - protein, 215 aa, Artificial Sequence
  AbD31988 - light chain
DIVLTQPPSVSGAPGQRVTISCSGSSSNIGSNAVWWYQQLPGTAPKLLIYDNNKRPSGVPDRFSGSKSGTSASLAITGLQAEDEADYYCQSWDLSLTSYVFGGGTKLTVLGQPKAAPSVTLFPPSSEELQANKATLVCLISDFYPGAVTVAWKADSSPVKAGVETTTPSKQSNNKYAASSYLSLTPEQWKSHRSYSCQVTHEGSTVEKTVAPTEA

SEQ ID NO: 8 - protein, 5 aa, Artificial Sequence
  AbD31988 heavy chain CDR1
SYAIS

SEQ ID NO: 9 - protein, 17 aa, Artificial Sequence
  AbD31988 heavy chain CDR2
RIIPIFGTANYAQKFQG

SEQ ID NO: 10 - protein, 16 aa, Artificial Sequence
  AbD31988 heavy chain CDR3
RIIPIFGTANYAQKFQ

SEQ ID NO: 11 - protein, 13 aa, Artificial Sequence
  AbD31988 light chain CDR1
SGSSSNIGSNAVW

SEQ ID NO: 12 - protein, 7 aa, Artificial Sequence
  AbD31988 light chain CDR2
DNNKRPS

SEQ ID NO: 13 - protein, 11 aa, Artificial Sequence
  AbD31988 light chain CDR3
QSWDLSLTSYV

SEQ ID NO: 14 - protein, 690 aa, Artificial Sequence
  AbD31998 Fd chain and tags
QVQLVQSGAEVKKPGASVKVSCKASGYTFSNYYMSWVRQAPGQGLEWMGWINPYNGVTNYAQKFQGRVTMTRDTSISTAYMELSRLRSEDTAVYYCARGLGSQFDYWGQGTLVTVSSASTKGPSVFPLAPSSKSTSGGTAALGCLVKDYFPEPVTVSWNSGALTSGVHTFPAVLQSSGLYSLSSVVTVPSSSLGTQTYICNVNHKPSNTKVDKKVEPKSEFKAEMPVLENRAAQGDITTPGGARRLTGDQTAALRDSLSDKPAKNIILLIGDGMGDSEITAARNYAEGAGGFFKGIDALPLTGQYTHYALNRKTGKPDYVTSSAASATAWSTGVKTYNGALGVDIHEKDHPTILEMAKAAGLATGNVSTAELQDATPAALVAHVTSRKCYGPSATSEKCPGNALEKGGKGSITEQLLNARADVTLGGGAKTFAETATAGEWQGKTLREQAQARGYQLVSDAASLNSVTEANQQKPLLGLFADGNMPVRWLGPKATYHGNIDKPAVTCTPNPQRNDSVPTLAQMTDKAIELLSKNEKGFFLQVEGASIDKQDHAANPCGQIGETVDLDEAVQRALEFAKKEGNTLVIVTADHAHASQIVAPDTKAPGLTQALNTKDGAVMVMSYGNSEEDSQEHTGSQLRIAAYGPHAANVVGLTDQTDLFYTMKAALGLKGAPDYKDDDDKGAPHHHHHH

SEQ ID NO: 15 - protein, 221 aa, Artificial Sequence
  AbD31998 heavy chain
QVQLVQSGAEVKKPGASVKVSCKASGYTFSNYYMSWVRQAPGQGLEWMGWINPYNGVTNYAQKFQGRVTMTRDTSISTAYMELSRLRSEDTAVYYCARGLGSQFDYWGQGTLVTVSSASTKGPSVFPLAPSSKSTSGGTAALGCLVKDYFPEPVTVSWNSGALTSGVHTFPAVLQSSGLYSLSSVVTVPSSSLGTQTYICNVNHKPSNTKVDKKVEPKSEF

SEQ ID NO: 16 - protein, 214 aa, Artificial Sequence
  AbD31998 light chain
DIALTQPASVSGSPGQSITISCTGTSSDVGKYNTVSWYQQHPGKAPKLMIYGVSKRPSGVSNRFSGSKSGNTASLTISGLQAEDEADYYCGSWDHLSYVFGGGTKLTVLGQPKAAPSVTLFPPSSEELQANKATLVCLISDFYPGAVTVAWKADSSPVKAGVETTTPSKQSNNKYAASSYLSLTPEQWKSHRSYSCQVTHEGSTVEKTVAPTEA

SEQ ID NO: 17 - protein, 5 aa, Artificial Sequence
  AbD31998 - heavy chain CDR1
NYYMS

SEQ ID NO: 18 - protein, 17 aa, Artificial Sequence
  AbD31998 heavy chain CDR2
WINPYNGVTNYAQKFQG

SEQ ID NO: 19 - protein, 8 aa, Artificial Sequence
  AbD31998 heavy chain CDR3
GLGSQFDY

SEQ ID NO: 20 - protein, 14 aa, Artificial Sequence
  AbD31998 light chain CDR1
TGTSSDVGKYNTVS

SEQ ID NO: 21 - protein, 7 aa, Artificial Sequence
  AbD31998 light chain CDR2
GVSKRPS

SEQ ID NO: 22 - protein, 9 aa, Artificial Sequence
  AbD31998 light chain CDR3
GSWDHLSYV

SEQ ID NO: 23 - protein, 691 aa, Artificial Sequence
  AbD31999 - Fd chain and tags
QVQLVQSGAEVKKPGASVKVSCKASGYTFTTYYMHWVRQAPGQGLEWMGRISPFSGNTNYAQKFQGRVTMTRDTSISTAYMELSRLRSEDTAVYYCARGIGPNWFDYWGQGTLVTVSSASTKGPSVFPLAPSSKSTSGGTAALGCLVKDYFPEPVTVSWNSGALTSGVHTFPAVLQSSGLYSLSSVVTVPSSSLGTQTYICNVNHKPSNTKVDKKVEPKSEFKAEMPVLENRAAQGDITTPGGARRLTGDQTAALRDSLSDKPAKNIILLIGDGMGDSEITAARNYAEGAGGFFKGIDALPLTGQYTHYALNRKTGKPDYVTSSAASATAWSTGVKTYNGALGVDIHEKDHPTILEMAKAAGLATGNVSTAELQDATPAALVAHVTSRKCYGPSATSEKCPGNALEKGGKGSITEQLLNARADVTLGGGAKTFAETATAGEWQGKTLREQAQARGYQLVSDAASLNSVTEANQQKPLLGLFADGNMPVRWLGPKATYHGNIDKPAVTCTPNPQRNDSVPTLAQMTDKAIELLSKNEKGFFLQVEGASIDKQDHAANPCGQIGETVDLDEAVQRALEFAKKEGNTLVIVTADHAHASQIVAPDTKAPGLTQALNTKDGAVMVMSYGNSEEDSQEHTGSQLRIAAYGPHAANVVGLTDQTDLFYTMKAALGLKGAPDYKDDDDKGAPHHHHHH

SEQ ID NO: 24 - protein, 222 aa, Artificial Sequence
  AbD31999 heavy chain
QVQLVQSGAEVKKPGASVKVSCKASGYTFTTYYMHWVRQAPGQGLEWMGRISPFSGNTNYAQKFQGRVTMTRDTSISTAYMELSRLRSEDTAVYYCARGIGPNWFDYWGQGTLVTVSSASTKGPSVFPLAPSSKSTSGGTAALGCLVKDYFPEPVTVSWNSGALTSGVHTFPAVLQSSGLYSLSSVVTVPSSSLGTQTYICNVNHKPSNTKVDKKVEPKSEF

SEQ ID NO: 25 - protein, 216 aa, Artificial Sequence
  AbD31999 light chain
DIVLTQPPSVSGAPGQRVTISCTGSSSNIGAGYDVHWYQQLPGTAPKLLIYYNYNRPSGVPDRFSGSKSGTSASLAITGLQAEDEADYYCQSWDSHLKSVVFGGGTKLTVLGQPKAAPSVTLFPPSSEELQANKATLVCLISDFYPGAVTVAWKADSSPVKAGVETTTPSKQSNNKYAASSYLSLTPEQWKSHRSYSCQVTHEGSTVEKTVAPTEA

SEQ ID NO: 26 - protein, 5 aa, Artificial Sequence
  AbD31999 heavy chain CDR1
TYYMH

SEQ ID NO: 27 - protein, 17 aa, Artificial Sequence
  AbD31999 heavy chain CDR2
RISPFSGNTNYAQKFQG

SEQ ID NO: 28 - protein, 9 aa, Artificial Sequence
  AbD31999 heavy chain CDR3
GIGPNWFDY

SEQ ID NO: 29 - protein, 14 aa, Artificial Sequence
  AbD31999 light chain CDR1
TGSSSNIGAGYDVH

SEQ ID NO: 30 - protein, 7 aa, Artificial Sequence
  AbD31999 - light chain CDR2
YNYNRPS

SEQ ID NO: 31 - protein, 11 aa, Artificial Sequence
  AbD31999 light chain CDR3
QSWDSHLKSVV

SEQ ID NO: 32 - DNA, 20 bp, Artificial Sequence
  CSSV ORF3 F-74 primer
ctgaagcgagtaggcaacaa

SEQ ID NO: 33 - DNA, 20 bp, Artificial Sequence
  CSSV ORF3 R-151 primer
cagtccaagggatggactct

SEQ ID NO: 34 - DNA, 20 bp, Artificial Sequence
  CSSV ORF3 P-129 probe
tccatcaggttgccatggca

SEQ ID NO: 35 - DNA, 24 bp, Artificial Sequence
  mTcCIR25 forward primer
cagataaggaaaggtggagtttgg

SEQ ID NO: 36 - DNA, 26 bp, Artificial Sequence
  mTcCIR25 reverse primer
caagaatgtctcctacattcactacg

SEQ ID NO: 37 - DNA, 25 bp, Artificial Sequence
  mTcCIR25 probe
ttcccgtaagcttcgtcccagatgc